European Patent Application EP 4 814 001 A1, published September 30, 2026. Title: Novel variant of GlnH protein and method for producing L-glutamic acid using the same. Applicant: DAESANG CORPORATION. The sequence listing filed with the application follows.

SEQUENCE LISTING (15 sequences)

SEQ ID NO: 1 - DNA, 1035 bp, Corynebacterium glutamicum
  source 1..1035: mol_type = genomic DNA
atgcacgcttttcgacgcccccctccactcaccacgcgagtcggcgctgcattgctggccgcaacgctgcttgcttcctgcactccaacacctgtggaaccggcagaaaccttgactgctttggatcccgatgccggtccaccactgccaccggattcttcgattgaagctcccggtgaaaaagagcccatagtggaagcaatagagaattggccaggttctttacgcccggatgatctgacccctgaggagcgggtacctggcatcgtcaaccggggtcgcatcattgtgggtgtggatcaatcgcaaaacttgctcagtttccgtgatccggtgactggtgagctgcgcggttttgaagtggaattagcgagggaaatttcccgtgacattttcggtgaccccaataaggtggatttccgattcgtcggctcgtccgaccgtctgcgttcccttgaccaaggtgatgtagatattgtgattcgttccgtcacgatcaccgacgaacgcgccaaattggtggaattttccacaccgtacctgcgcacccaaacccgcatgttgaccatggaatcttcaggaatcacgtccatcgcagatctacccggccacaccatttgtgtcaccgatggctccacttcattgcagcgagcccgcaccattgcgccggaggcctcaatcttaaaaactcgcaattggtccgattgtctcatggcgttgcagcagcatcaggctcaggtcattttgggcgatgatgtcattttgtccggcatcgcagcacaggatccctacaccgagattcttgatacctccctcgattcccattcctatggagtggcagcggcatcgaccactgctgaaacagactcttcggggttgattcggcaggtaaactacacaattgaacggatccgcacagaccgcatgtggtggacaatgttcgacgattggttcggaccttatctctggtcctacggtccaccacagctgcagtacatgccagaggaagaagggacagaaaacgatgaaggataa

SEQ ID NO: 2 - protein, 344 aa, Corynebacterium glutamicum
MHAFRRPPPLTTRVGAALLAATLLASCTPTPVEPAETLTALDPDAGPPLPPDSSIEAPGEKEPIVEVIENWPGSLRPDDLTPEERVPGIVNRGRIIVGVDQSQNLLSFRDPVTGELRGFEVELAREISRDIFGDPNKVDFRFVGSSDRLRSLDQGDVDIVIRSVTITDERAKLVEFSTPYLRTQTRMLTMESSGITSIADLPGHTICVTDGSTSLQRARTIAPEASILKTRNWSDCLMALQQHQAQVILGDDVILSGIAAQDPYTEILDTSLDSHSYGVAAASTTAETDSSGLIRQVNYTIERIRTDRMWWTMFDDWFGPYLWSYGPPQLQYMPEEEGTENDEG

SEQ ID NO: 3 - DNA, 1035 bp, synthetic construct
  source 1..1035: mol_type = other DNA
atgcacgcttttcgacgcccccctccactcatcacgcgagtcggcgctgcattgctggccgcaacgctgcttgcttcctgcactccaacacctgtggaaccggcagaaaccttgactgctttggatcccgatgccggtccaccactgccaccggattcttcgattgaagctcccggtgaaaaagagcccatagtggaagcaatagagaattggccaggttctttacgcccggatgatctgacccctgaggagcgggtacctggcatcgtcaaccggggtcgcatcattgtgggtgtggatcaatcgcaaaacttgctcagtttccgtgatccggtgactggtgagctgcgcggttttgaagtggaattagcgagggaaatttcccgtgacattttcggtgaccccaataaggtggatttccgattcgtcggctcgtccgaccgtctgcgttcccttgaccaaggtgatgtagatattgtgattcgttccgtcacgatcaccgacgaacgcgccaaattggtggaattttccacaccgtacctgcgcacccaaacccgcatgttgaccatggaatcttcaggaatcacgtccatcgcagatctacccggccacaccatttgtgtcaccgatggctccacttcattgcagcgagcccgcaccattgcgccggaggcctcaatcttaaaaactcgcaattggtccgattgtctcatggcgttgcagcagcatcaggctcaggtcattttgggcgatgatgtcattttgtccggcatcgcagcacaggatccctacaccgagattcttgatacctccctcgattcccattcctatggagtggcagcggcatcgaccactgctgaaacagactcttcggggttgattcggcaggtaaactacacaattgaacggatccgcacagaccgcatgtggtggacaatgttcgacgattggttcggaccttatctctggtcctacggtccaccacagctgcagtacatgccagaggaagaagggacagaaaacgatgaaggataa

SEQ ID NO: 4 - protein, 344 aa, synthetic construct
MHAFRRPPPLITRVGAALLAATLLASCTPTPVEPAETLTALDPDAGPPLPPDSSIEAPGEKEPIVEVIENWPGSLRPDDLTPEERVPGIVNRGRIIVGVDQSQNLLSFRDPVTGELRGFEVELAREISRDIFGDPNKVDFRFVGSSDRLRSLDQGDVDIVIRSVTITDERAKLVEFSTPYLRTQTRMLTMESSGITSIADLPGHTICVTDGSTSLQRARTIAPEASILKTRNWSDCLMALQQHQAQVILGDDVILSGIAAQDPYTEILDTSLDSHSYGVAAASTTAETDSSGLIRQVNYTIERIRTDRMWWTMFDDWFGPYLWSYGPPQLQYMPEEEGTENDEG

SEQ ID NO: 5 - DNA, 1035 bp, synthetic construct
  source 1..1035: mol_type = other DNA
atgcacgcttttcgacgcccccctccactcaccacgcgagtcggcgctgcattgctggccgcaacgctgcttgcttcctgcactccaacacctgtggaaccggcagaaaccttgactgctttggatcccgatgccggtccaccactgccaccggattcttcgattgaagctcccggtgaaaaagagcccatagtggaagcaatagagaattggccaggttctttacgcccggatgatctgacccctgaggagcgggtacctggcatcgtcaaccggggtcgcatcattgtgggtgtggatcaatcgcaaaacttgctcagtttccgtgatccggtgactggtgagctgcgcggttttgaagtggaattagcgagggaaatttcccgtgacattttcggtgaccccaataaggtggatttccgattcgtcggctcgtccgaccgtctgcgttcccttgaccaaggtgatgtagatattgtgattcgttccgtcgcgatcaccgacgaacgcgccaaattggtggaattttccacaccgtacctgcgcacccaaacccgcatgttgaccatggaatcttcaggaatcacgtccatcgcagatctacccggccacaccatttgtgtcaccgatggctccacttcattgcagcgagcccgcaccattgcgccggaggcctcaatcttaaaaactcgcaattggtccgattgtctcatggcgttgcagcagcatcaggctcaggtcattttgggcgatgatgtcattttgtccggcatcgcagcacaggatccctacaccgagattcttgatacctccctcgattcccattcctatggagtggcagcggcatcgaccactgctgaaacagactcttcggggttgattcggcaggtaaactacacaattgaacggatccgcacagaccgcatgtggtggacaatgttcgacgattggttcggaccttatctctggtcctacggtccaccacagctgcagtacatgccagaggaagaagggacagaaaacgatgaaggataa

SEQ ID NO: 6 - protein, 344 aa, synthetic construct
MHAFRRPPPLTTRVGAALLAATLLASCTPTPVEPAETLTALDPDAGPPLPPDSSIEAPGEKEPIVEVIENWPGSLRPDDLTPEERVPGIVNRGRIIVGVDQSQNLLSFRDPVTGELRGFEVELAREISRDIFGDPNKVDFRFVGSSDRLRSLDQGDVDIVIRSVAITDERAKLVEFSTPYLRTQTRMLTMESSGITSIADLPGHTICVTDGSTSLQRARTIAPEASILKTRNWSDCLMALQQHQAQVILGDDVILSGIAAQDPYTEILDTSLDSHSYGVAAASTTAETDSSGLIRQVNYTIERIRTDRMWWTMFDDWFGPYLWSYGPPQLQYMPEEEGTENDEG

SEQ ID NO: 7 - DNA, 1035 bp, synthetic construct
  source 1..1035: mol_type = other DNA
atgcacgcttttcgacgcccccctccactcatcacgcgagtcggcgctgcattgctggccgcaacgctgcttgcttcctgcactccaacacctgtggaaccggcagaaaccttgactgctttggatcccgatgccggtccaccactgccaccggattcttcgattgaagctcccggtgaaaaagagcccatagtggaagcaatagagaattggccaggttctttacgcccggatgatctgacccctgaggagcgggtacctggcatcgtcaaccggggtcgcatcattgtgggtgtggatcaatcgcaaaacttgctcagtttccgtgatccggtgactggtgagctgcgcggttttgaagtggaattagcgagggaaatttcccgtgacattttcggtgaccccaataaggtggatttccgattcgtcggctcgtccgaccgtctgcgttcccttgaccaaggtgatgtagatattgtgattcgttccgtcgcgatcaccgacgaacgcgccaaattggtggaattttccacaccgtacctgcgcacccaaacccgcatgttgaccatggaatcttcaggaatcacgtccatcgcagatctacccggccacaccatttgtgtcaccgatggctccacttcattgcagcgagcccgcaccattgcgccggaggcctcaatcttaaaaactcgcaattggtccgattgtctcatggcgttgcagcagcatcaggctcaggtcattttgggcgatgatgtcattttgtccggcatcgcagcacaggatccctacaccgagattcttgatacctccctcgattcccattcctatggagtggcagcggcatcgaccactgctgaaacagactcttcggggttgattcggcaggtaaactacacaattgaacggatccgcacagaccgcatgtggtggacaatgttcgacgattggttcggaccttatctctggtcctacggtccaccacagctgcagtacatgccagaggaagaagggacagaaaacgatgaaggataa

SEQ ID NO: 8 - protein, 344 aa, synthetic construct
MHAFRRPPPLITRVGAALLAATLLASCTPTPVEPAETLTALDPDAGPPLPPDSSIEAPGEKEPIVEVIENWPGSLRPDDLTPEERVPGIVNRGRIIVGVDQSQNLLSFRDPVTGELRGFEVELAREISRDIFGDPNKVDFRFVGSSDRLRSLDQGDVDIVIRSVAITDERAKLVEFSTPYLRTQTRMLTMESSGITSIADLPGHTICVTDGSTSLQRARTIAPEASILKTRNWSDCLMALQQHQAQVILGDDVILSGIAAQDPYTEILDTSLDSHSYGVAAASTTAETDSSGLIRQVNYTIERIRTDRMWWTMFDDWFGPYLWSYGPPQLQYMPEEEGTENDEG

SEQ ID NO: 9 - DNA, 5719 bp, synthetic construct
  source 1..5719: mol_type = other DNA
tgccgcaagcactcagggcgcaagggctgctaaaggaagcggaacacgtagaaagccagtccgcagaaacggtgctgaccccggatgaatgtcagctactgggctatctggacaagggaaaacgcaagcgcaaagagaaagcaggtagcttgcagtgggcttacatggcgatagctagactgggcggttttatggacagcaagcgaaccggaattgccagctggggcgccctctggtaaggttgggaagccctgcaaagtaaactggatggctttcttgccgccaaggatctgatggcgcaggggatcaagatctgatcaagagacaggatgaggatcgtttcgcatgattgaacaagatggattgcacgcaggttctccggccgcttgggtggagaggctattcggctatgactgggcacaacagacaatcggctgctctgatgccgccgtgttccggctgtcagcgcaggggcgcccggttctttttgtcaagaccgacctgtccggtgccctgaatgaactccaagacgaggcagcgcggctatcgtggctggccacgacgggcgttccttgcgcagctgtgctcgacgttgtcactgaagcgggaagggactggctgctattgggcgaagtgccggggcaggatctcctgtcatctcaccttgctcctgccgagaaagtatccatcatggctgatgcaatgcggcggctgcatacgcttgatccggctacctgcccattcgaccaccaagcgaaacatcgcatcgagcgagcacgtactcggatggaagccggtcttgtcgatcaggatgatctggacgaagagcatcaggggctcgcgccagccgaactgttcgccaggctcaaggcgcggatgcccgacggcgaggatctcgtcgtgacccatggcgatgcctgcttgccgaatatcatggtggaaaatggccgcttttctggattcatcgactgtggccggctgggtgtggcggaccgctatcaggacatagcgttggctacccgtgatattgctgaagagcttggcggcgaatgggctgaccgcttcctcgtgctttacggtatcgccgctcccgattcgcagcgcatcgccttctatcgccttcttgacgagttcttctgagcgggactctggggttcgctagaggatcgatcctttttaacccatcacatatacctgccgttcactattatttagtgaaatgagatattatgatattttctgaattgtgattaaaaaggcaactttatgcccatgcaacagaaactataaaaaatacagagaatgaaaagaaacagatagattttttagttctttaggcccgtagtctgcaaatccttttatgattttctatcaaacaaaagaggaaaatagaccagttgcaatccaaacgagagtctaatagaatgaggtcgaaaagtaaatcgcgcgggtttgttactgataaagcaggcaagacctaaaatgtgtaaagggcaaagtgtatactttggcgtcaccccttacatattttaggtctttttttattgtgcgtaactaacttgccatcttcaaacaggagggctggaagaagcagaccgctaacacagtacataaaaaaggagacatgaacgatgaacatcaaaaagtttgcaaaacaagcaacagtattaacctttactaccgcactgctggcaggaggcgcaactcaagcgtttgcgaaagaaacgaaccaaaagccatataaggaaacatacggcatttcccatattacacgccatgatatgctgcaaatccctgaacagcaaaaaaatgaaaaatatcaagtttctgaatttgattcgtccacaattaaaaatatctcttctgcaaaaggcctggacgtttgggacagctggccattacaaaacgctgacggcactgtcgcaaactatcacggctaccacatcgtctttgcattagccggagatcctaaaaatgcggatgacacatcgatttacatgttctatcaaaaagtcggcgaaacttctattgacagctggaaaaacgctggccgcgtctttaaagacagcgacaaattcgatgcaaatgattctatcctaaaagaccaaacacaagaatggtcaggttcagccacatttacatctgacggaaaaatccgtttattctacactgatttctccggtaaacattacggcaaacaaacactgacaactgcacaagttaacgtatcagcatcagacagctctttgaacatcaacggtgtagaggattataaatcaatctttgacggtgacggaaaaacgtatcaaaatgtacagcagttcatcgatgaaggcaactacagctcaggcgacaaccatacgctgagagatcctcactacgtagaagataaaggccacaaatacttagtatttgaagcaaacactggaactgaagatggctaccaaggcgaagaatctttatttaacaaagcatactatggcaaaagcacatcattcttccgtcaagaaagtcaaaaacttctgcaaagcgataaaaaacgcacggctgagttagcaaacggcgctctcggtatgattgagctaaacgatgattacacactgaaaaaagtgatgaaaccgctgattgcatctaacacagtaacagatgaaattgaacgcgcgaacgtctttaaaatgaacggcaaatggtacctgttcactgactcccgcggatcaaaaatgacgattgacggcattacgtctaacgatatttacatgcttggttatgtttctaattctttaactggcccatacaagccgctgaacaaaactggccttgtgttaaaaatggatcttgatcctaacgatgtaacctttacttactcacacttcgctgtacctcaagcgaaaggaaacaatgtcgtgattacaagctatatgacaaacagaggattctacgcagacaaacaatcaacgtttgcgccgagcttcctgctgaacatcaaaggcaagaaaacatctgttgtcaaagacagcatccttgaacaaggacaattaacagttaacaaataaaaacgcaaaagaaaatgccgatgggtaccgagcgaaatgaccgaccaagcgacgcccaacctgccatcacgagatttcgattccaccgccgccttctatgaaaggttgggcttcggaatcgttttccgggacgccctcgcggacgtgctcatagtccacgacgcccgtgattttgtagccctggccgacggccagcaggtaggccgacaggctcatgccggccgccgccgccttttcctcaatcgctcttcgttcgtctggaaggcagtacaccttgataggtgggctgcccttcctggttggcttggtttcatcagccatccgcttgccctcatctgttacgccggcggtagccggccagcctcgcagagcaggattcccgttgagcaccgccaggtgcgaataagggacagtgaagaaggaacacccgctcgcgggtgggcctacttcacctatcctgcccggctgacgccgttggatacaccaaggaaagtctacacgaaccctttggcaaaatcctgtatatcgtgcgaaaaaggatggatataccgaaaaaatcgctataatgaccccgaagcagggttatgcagcggaaaagcgctgcttccctgctgttttgtggaatatctaccgactggaaacaggcaaatgcaggaaattactgaactgaggggacaggcgagagacgatgccaaagagctcctgaaaatctcgataactcaaaaaatacgcccggtagtgatcttatttcattatggtgaaagttggaacctcttacgtgccgatcaacgtctcattttcgccaaaagttggcccagggcttcccggtatcaacagggacaccaggatttatttattctgcgaagtgatcttccgtcacaggtatttattcggcgcaaagtgcgtcgggtgatgctgccaacttactgatttagtgtatgatggtgtttttgaggtgctccagtggcttctgtttctatcagctcctgaaaatctcgataactcaaaaaatacgcccggtagtgatcttatttcattatggtgaaagttggaacctcttacgtgccgatcaacgtctcattttcgccaaaagttggcccagggcttcccggtatcaacagggacaccaggatttatttattctgcgaagtgatcttccgtcacaggtatttattcggcgcaaagtgcgtcgggtgatgctgccaacttactgatttagtgtatgatggtgtttttgaggtgctccagtggcttctgtttctatcagggctggatgatcctccagcgcggggatctcatgctggagttcttcgcccaccccaaaaggatctaggtgaagatcctttttgataatctcatgaccaaaatcccttaacgtgagttttcgttccactgagcgtcagaccccgtagaaaagatcaaaggatcttcttgagatcctttttttctgcgcgtaatctgctgcttgcaaacaaaaaaaccaccgctaccagcggtggtttgtttgccggatcaagagctaccaactctttttccgaaggtaactggcttcagcagagcgcagataccaaatactgttcttctagtgtagccgtagttaggccaccacttcaagaactctgtagcaccgcctacatacctcgctctgctaatcctgttaccagtggctgctgccagtggcgataagtcgtgtcttaccgggttggactcaagacgatagttaccggataaggcgcagcggtcgggctgaacggggggttcgtgcacacagcccagcttggagcgaacgacctacaccgaactgagatacctacagcgtgagctatgagaaagcgccacgcttcccgaagggagaaaggcggacaggtatccggtaagcggcagggtcggaacaggagagcgcacgagggagcttccagggggaaacgcctggtatctttatagtcctgtcgggtttcgccacctctgacttgagcgtcgatttttgtgatgctcgtcaggggggcggagcctatggaaaaacgccagcaacgcggcctttttacggttcctggccttttgctggccttttgctcacatgttctttcctgcgttatcccctgattctgtggataaccgtattaccgcctttgagtgagctgataccgctcgccgcagccgaacgaccgagcgcagcgagtcagtgagcgaggaagcggaagagcgcccaatacgcaaaccgcctctccccgcgcgttggccgattcattaatgcagctggcacgacaggtttcccgactggaaagcgggcagtgagcgcaacgcaattaatgtgagttagctcactcattaggcaccccaggctttacactttatgcttccggctcgtatgttgtgtggaattgtgagcggataacaatttcacacaggaaacagctatgacatgattacgccaagcttgcatgcctgcaggtcgactctagaggatccccgggtaccgagctcgaattcactggccgtcgttttacaacgtcgtgactgggaaaaccctggcgttacccaacttaatcgccttgcagcacatccccctttcgccagctggcgtaatagcgaagaggcccgcaccgatcgcccttcccaacagttgcgcagcctgaatggcgaatggcgataagctagcttcacgc

SEQ ID NO: 10 - DNA, 20 bp, synthetic construct
  source 1..20: mol_type = other DNA
gagacgttgtcgttggtgcg

SEQ ID NO: 11 - DNA, 18 bp, synthetic construct
  source 1..18: mol_type = other DNA
cgcgtgatgagtggaggg

SEQ ID NO: 12 - DNA, 18 bp, synthetic construct
  source 1..18: mol_type = other DNA
ccctccactcatcacgcg

SEQ ID NO: 13 - DNA, 20 bp, synthetic construct
  source 1..20: mol_type = other DNA
gtcggtgatcgcgacggaac

SEQ ID NO: 14 - DNA, 20 bp, synthetic construct
  source 1..20: mol_type = other DNA
gttccgtcgcgatcaccgac

SEQ ID NO: 15 - DNA, 24 bp, synthetic construct
  source 1..24: mol_type = other DNA
ttatccttcatcgttttctgtccc